European Patent Application EP 4 810 617 A1, published September 23, 2026. Title: 基于I型内含子的RNA体外环化与滚环翻译的方法及其应用. Applicant: 复旦大学. The sequence listing filed with the application follows.

SEQUENCE LISTING (62 sequences)

SEQ ID NO: 1 - DNA, 19 bp, synthetic construct
  source 1..19: mol_type = other DNA
taatacgactcactatagg

SEQ ID NO: 2 - DNA, 35 bp, synthetic construct
  source 1..35: mol_type = other DNA
aagtatattgattagttttggagtactcgtaaggt

SEQ ID NO: 3 - skipped

SEQ ID NO: 4 - DNA, 741 bp, synthetic construct
  source 1..741: mol_type = other DNA
ttaaaacagcctgtgggttgatcccacccacaggcccattgggcgctagcactctggtatcacggtacctttgtgcgcctgttttataccccctcccccaactgtaacttagaagtaacacacaccgatcaacagtcagcgtggcacaccagccacgttttgatcaagcacttctgttaccccggactgagtatcaatagactgctcacgcggttgaaggagaaagcgttcgttatccggccaactacttcgaaaaacctagtaacaccgtggaagttgcagagtgtttcgctcagcactaccccagtgtagatcaggtcgatgagtcaccgcattccccacgggcgaccgtggcggtggctgcgttggcggcctgcccatggggaaacccatgggacgctctaatacagacatggtgcgaagagtctattgagctagttggtagtcctccggcccctgaatgcggctaatcctaactgcggagcacacaccctcaagccagagggcagtgtgtcgtaacgggcaactctgcagcggaaccgactactttgggtgtccgtgtttcattttattcctatactggctgcttatggtgacaattgagagatcgttaccatatagctattggattggccatccggtgactaatagagctattatatatccctttgttgggtttataccacttagcttgaaagaggttaaaacattacaattcattgttaagttgaatacagcaaa

SEQ ID NO: 5 - DNA, 720 bp, synthetic construct
  source 1..720: mol_type = other DNA
atggtgagcaagggcgaggagctgttcaccggggtggtgcccatcctggtcgagctggacggcgacgtaaacggccacaagttcagcgtgtccggcgagggcgagggcgatgccacctacggcaagctgaccctgaagttcatctgcaccaccggcaagctgcccgtgccctggcccaccctcgtgaccaccctgacctacggcgtgcagtgcttcagccgctaccccgaccacatgaagcagcacgacttcttcaagtccgccatgcccgaaggctacgtccaggagcgcaccatcttcttcaaggacgacggcaactacaagacccgcgccgaggtgaagttcgagggcgacaccctggtgaaccgcatcgagctgaagggcatcgacttcaaggaggacggcaacatcctggggcacaagctggagtacaactacaacagccacaacgtctatatcatggccgacaagcagaagaacggcatcaaggtgaacttcaagatccgccacaacatcgaggacggcagcgtgcagctcgccgaccactaccagcagaacacccccatcggcgacggccccgtgctgctgcccgacaaccactacctgagcacccagtccgccctgagcaaagaccccaacgagaagcgcgatcacatggtcctgctggagttcgtgaccgccgccgggatcactctcggcatggacgagctgtacaagtaa

SEQ ID NO: 6 - DNA, 390 bp, synthetic construct
  source 1..390: mol_type = other DNA
ctctctaaatagcaatatttacctttggagggaaaagttatcaggcatgcacctggtagctagtctttaaaccaatagattgcatcggtttaaaaggcaagaccgtcaaattgcgggaaaggggtcaacagccgttcagtaccaagtctcaggggaaactttgagatggccttgcaaagggtatggtaataagctgacggacatggtcctaaccacgcagccaagtcctaagtcaacagatcttctgttgatatggatgcagttcacagactaaatgtcggtcggggaagatgtattcttctcataagatatagtcggacctctccttaatgggagctagcggatgaagtgatgcaacactggagccgctgggaactaatttgtatgcga

SEQ ID NO: 7 - DNA, 425 bp, synthetic construct
  source 1..425: mol_type = other DNA
ctctctaaatagcaatatttacctttggagggaaaagttatcaggcatgcacctggtagctagtctttaaaccaatagattgcatcggtttaaaaggcaagaccgtcaaattgcgggaaaggggtcaacagccgttcagtaccaagtctcaggggaaactttgagatggccttgcaaagggtatggtaataagctgacggacatggtcctaaccacgcagccaagtcctaagtcaacagatcttctgttgatatggatgcagttcacagactaaatgtcggtcggggaagatgtattcttctcataagatatagtcggacctctccttaatgggagctagcggatgaagtgatgcaacactggagccgctgggaactaatttgtatgcgaaagtatattgattagttttggagtactcgtaaggt

SEQ ID NO: 8 - DNA, 419 bp, synthetic construct
  source 1..419: mol_type = other DNA
ctctctaaatagcaatatttacctttggagggaaaagttatcaggcatgcacctggtagctagtctttaaaccaatagattgcatcggtttaaaaggcaagaccgtcaaattgcgggaaaggggtcaacagccgttcagtaccaagtctcaggggaaactttgagatggccttgcaaagggtatggtaataagctgacggacatggtcctaaccacgcagccaagtcctaagtcaacagatcttctgttgatatggatgcagttcacagactaaatgtcggtcggggaagatgtattcttctcataagatatagtcggacctctccttaatgggagctagcggatgaagtgatgcaacactggagccgctgggaactaatttgtatgcgaaagtatattgattagttttggagtactcg

SEQ ID NO: 9 - RNA, 39 nt, synthetic construct
  source 1..39: mol_type = other RNA
tgtttaggttcgcttttctgttttatttgtttcgaaaac

SEQ ID NO: 10 - RNA, 140 nt, synthetic construct
  source 1..140: mol_type = other RNA
gtgaagattgaccatctcacaaaagctgttacgtgcttgtaacacactactcactcgttttgtattcgagaagtagttgcaacaacggttccctcattgcctgacaagctgagggccacccttctatccccaccgccatc

SEQ ID NO: 11 - RNA, 288 nt, synthetic construct
  source 1..288: mol_type = other RNA
atgcaagagaaaagtttggtagacacacacggcgggacgtgttgctagagctgccactctgcccgagatggatcgatattaaccatctttggcaacagcgtgtgtgatcgaccaaacctagtaattgcgtagcatccgactgtaacctgttctctgctgaatgcgagggtggcctcgtgatcccaaaccataaaagaaaccaacttgttggtggaagggcttggaagtaggatcaaccactgtttattaattaggggtgagagtattcactgtactctttccccgccc

SEQ ID NO: 12 - RNA, 274 nt, synthetic construct
  source 1..274: mol_type = other RNA
agtaagtagcctaacctgctgcagcaggaagtattctaggtagtatagtaactctttcttcaacttcttacttagaaaaacacaaaaatacccccagctcgcttttgttttgagctgtgttagggaccaaaaacggcgactcatccgtcctgagtggcctctggtgtggaaaccagagagtcttgcggtaaccaacgaaatctcttcggagtgggtgttggggaccaccaaatgaagaaaatagcccctccctcgcgcaggggggggccagccc

SEQ ID NO: 13 - RNA, 177 nt, synthetic construct
  source 1..177: mol_type = other RNA
tgaaacagcagattacttttatttatgcatttaatggattgaagaaaagaaccttttttttctctctctctctgcaactgcagtaagggaggggagttggatatacctcgcctaatatctcctgggttgacaccatcattattgtttattcttgtgctccaaaagccgagtcctctg

SEQ ID NO: 14 - RNA, 284 nt, synthetic construct
  source 1..284: mol_type = other RNA
gtttgtattgtatgggcctccgtgaagttaggggcagtggaaacgtcggtctagccagccgtcccctgggtagtgtgctctgtctatgtacaccactactcggtttccacaaacgatcggactcccaatatagtgtacattatgttgattgcttctttctacctatataatatctcctctcatctctcctctacgcttggaatccataaaatccttcgggtgggcttggatttcgggtacttgtttgaaattccctcacgaccgccatagttgtgaggcagccc

SEQ ID NO: 15 - RNA, 284 nt, synthetic construct
  source 1..284: mol_type = other RNA
gtgctgcctcgtctgaggggacaggaggatcaccctcttcgtcgcttcggccagtgtgtcgggctgggccctgacaagccacctgaggagaggctcggagccgggcccggaccccggcgattgccgcccgcttctctctagtctcacgaggggtttcccgcctcgcacccccacctctggacttgcctttccttctcttctccgcgtgtggagggagccagcgcttaggccggagcgagcctgggggccgcccgccgtgaagacatcgcggggaccgattcacc

SEQ ID NO: 16 - RNA, 134 nt, synthetic construct
  source 1..134: mol_type = other RNA
tctagagccaccgtccagggagcaggtagctgctgggctccggggacactttgcgttcgggctgggagcgtgctttccacgacggtgacacgcttccctggattggcagccagactgccttccgggtcactgcc

SEQ ID NO: 17 - RNA, 443 nt, synthetic construct
  source 1..443: mol_type = other RNA
ttggttcttttaagtgtagcctccacccgagttgcaagaggggaacacgcagtctcgccgaccctgttggcaaacagtaaaattgcaaaaaatagagtgctaggagtagttcccgtacccgcgggagcaagaccctactacagtagacgaaccggcatcggaccctgggaaacaggtacctagcgtattaataggtcgctagaaatcgggcgggcttcaccttcgggtaacccgccgtcgagagggaaaacctctgtgtggttgtgcgcacgtcgttgtcggaagactctcactgttgtagttatttcctttttcttttaggtaggagcacttgctcagagggcgcatacctctggtaaaacaaaattggcccctgagagtagaaaactcaggttaataaaacaggagaatatttacctagtcgtataacggctaggtacccc

SEQ ID NO: 18 - RNA, 283 nt, synthetic construct
  source 1..283: mol_type = other RNA
ttatttgtatatgttatgtataattataatcatgcaatggcacatgtagttcccctaacctctcagtaggagtcaagccctgatgcgccaacatccagaagggggtaaagctgagtcggtgcaaggaaccttgttagccctaagaaaaacccaaaaacagagtgcatagtttagcttttgtgttgtaggagccagagaccaaagatccagacaactggtgagggcggtcgatggtgcgaagtaaattagaaaggggggcgtttacccacgtcctcccttgccc

SEQ ID NO: 19 - RNA, 326 nt, synthetic construct
  source 1..326: mol_type = other RNA
acctgcccaaggttatcacaggctaggaccggcctgataaaggtccgacttgatgtgcagcttcttaggtgcatctcgtatagaagcgctctggacatgacacctttgagacagaccgtacagcagtcacacgggacgccacaccacctttgcagaggtgcccttgggaaaccaatggtgtggggtgacactgattagtcgttaacggtgtactaatccagagtagttcagtgcaggggaaacccgggccgtaagcacgtggaactatataacttaatctcgctgagaagattgggggggattcatgaaatcccctcaccaggccc

SEQ ID NO: 20 - RNA, 234 nt, synthetic construct
  source 1..234: mol_type = other RNA
acactaagagttactgccaccaaaagaggataatcagaccacttgtagtttgctgccacaaactggttgacaagttaatgcctctctcttagttagtaagccggattcaagtagggaatgtggagggagatgccatggtggcatcagagcagacctggaaatactcttcggaggggcgccagaactgcactaaacacttgttatcaggggactgttgaggagtctccccgcccg

SEQ ID NO: 21 - RNA, 351 nt, synthetic construct
  source 1..351: mol_type = other RNA
gttcgctgaaacgagtgtaaatctggcatagcatacaggttactcttgttgggttctagatgttatgatgacgagtcggttcgggctccgcactaggtttggtcacctaggggatggagatatggaaagggtctcgtgtgctgttagacggtcgtaagacgcgcttgcaacatgggcctatgaccggataagtcatagcaatactagccaacatgaataggattcctgtttacgaaagttagatgtcacttgtggaaacggacccagacacggttgatctcaccttcgggggggctatagagatcgctggaagcactaccggacaaccggaacattgcagaaatgcagccc

SEQ ID NO: 22 - RNA, 235 nt, synthetic construct
  source 1..235: mol_type = other RNA
aggaagatgcttgggggtgttcccctaaagttcagaatggtctatcagggagcaggcacttttccggctttggcgagtcgtctccacttgtatacgaacagtgaggggaaaagttatctgatagaagaatgaaccatggacaaggacactctaaaccaccactaagaagctatagggaaaccttgctgagggcagtgagtggtcgtaccagaacgaatatggctttgccccgccc

SEQ ID NO: 23 - RNA, 246 nt, synthetic construct
  source 1..246: mol_type = other RNA
acgggatgagcttctgggggctgccaccctcgcctcatgcgcattgcctgctctgggcgcatgtggaagctgatatagttgagagcttcgtggaaggatgtggaaaccaagggagggagatatccagggaggatgtcggagttgtaaggataaaatacctaagcttcatcaggttaggttgggcttccgatgcaacaaaacaccagtagataaatagggggggatccaggggatccttctccgccc

SEQ ID NO: 24 - RNA, 221 nt, synthetic construct
  source 1..221: mol_type = other RNA
gacaaactctccgcctaatgtctgatgatgtgaggaacgtggactgtgatgtggtggtgcggtaccatggctggtcaccatggtaatgcgtagggcaacacagttcattaagactcactgatgatggcactaggcacggttcacccccatccttcgggagggctatagggggtgaccgggttacaccaccggaagaccggaacattgcctttgggcagccc

SEQ ID NO: 25 - RNA, 323 nt, synthetic construct
  source 1..323: mol_type = other RNA
atctcgccttaggtttacggttacccgagcttcgcctgaaacggcgttcctctaattccttcctggttctttccctccacggctcgcgtgttctgcggaactgcatctgcttcacttccttctttttccctctgtggtggtacgaccaatgggtggctcccattgactgcgtaggacatggaaaaagattgagtggagtgcacgaagcgtcgcaagatcgctgcctgacgaggtccagccaatcaaataccaaacatctggtttgggggcggattggctgtatgtcatgtaagtttgaggggttctatcggagccccccgccc

SEQ ID NO: 26 - RNA, 246 nt, synthetic construct
  source 1..246: mol_type = other RNA
ggaaagccactgcggtggggtcagtctcctggtgcgccaacacccagaaggggagacaacttcagtggttcaaaacccgatgcttcgtgtaagcctagaaaaatccaaaaacagagtgctactgctttcagtgtgcgagctttatttgctcacttcctccgtcgataaaatcccgaattttcgggtgggcttcggcggacatccttaatgaagaacgggggggtaacccacccccctgatctgccc

SEQ ID NO: 27 - RNA, 706 nt, synthetic construct
  source 1..706: mol_type = other RNA
ggcttcgcttcccgccggaagaccgcggcggttctgttcctcccacaggagtacggcaacaacccaccttgggaaagtggggaccccagcactaactcctttaactaggcgggcgtgctggttacagtaggaggggacagtgcgcatcaaaactgagccccaccacaactctcatccacagggtggttgggacgcaggtgtcggagggatcgccagccctcaggatagtgagctcccgcagagggataagctatctccctgcgacgtagtggtagaacacgtgggataggggatgaccttgtcgaccggttatcggtcccctgctccttcgagctggcaaggcgcccaaaggttctacactgctactaaagttggtggtggatgtctcgcccaaaaagatcataaacgcgcgggataaggtccctttccaccttcgccgggtaaggctagagtcagcgctgcatgactataacttgcggccgatccagttgcacgactggtggtccccctcagtgtcttggttgtctgccaagtgggcggtggtcggattccaccacaccctgccacgaggtgcgtggagacttggccagtctaggctcgtcgtaattagttgcagcgacgttaatcaacccgtccgggcatacaataggaccggttgtgcttcttcctccctttcttagccagggtggttacctccctggcgccc

SEQ ID NO: 28 - RNA, 236 nt, synthetic construct
  source 1..236: mol_type = other RNA
gagggcagtcaccctaccttctgccagaggttcccggaggagtagtgatcctttgggggtgattcatagctaggaaaggtcggagagttgggaggaggccaactgggggaggtgctaggagcaccagatgcagcagagcaaaaatccgggtttcatcgcctggtgcgggcgctcaatgctgctaacacgttcctgaaggaagaaaggtttcggtcgatggagaccttaacccgccc

SEQ ID NO: 29 - RNA, 263 nt, synthetic construct
  source 1..263: mol_type = other RNA
caatatgcacgagctgtcttgtaacacagcaatggagtaagtgtactctggtagcaatgggtggggtcgatttcctacgtctagctttggccggctagcgtctctcgtagtggggaaataactcattgagaccagctcagaacgctgacattgtctgtgtttggatagagggcttggggaaaactccgtaaggaggggcgcccgagagcctagtaacaccaaatttataaactaggggggaccgttaaggtctcccccgcccc

SEQ ID NO: 30 - RNA, 351 nt, synthetic construct
  source 1..351: mol_type = other RNA
gtttgtggagatgagtgtaaatctggcatagcatacaggttactcttgttgggttctggatgttaggatgacgagtcgactcgggctccgcactaggtttggtcgcctaggggatggagatatggaaagggtctcgtgtggtatcagtcggtcgaaagacgcgcttccaacatgggcctatggtcggataagtcttagcaataccagccagcatgaattggattcctgtttacgaaagttaggtgtcacttgtggaagcggacccagacacggttgatctcacccttcggggggctatagagatcgctggaagcactaccggacaaccggaacattgcagaaatgcagccc

SEQ ID NO: 31 - RNA, 251 nt, synthetic construct
  source 1..251: mol_type = other RNA
tacggtaatagtgtagtcttctcatcttagtagttagctctctcttatattaagaaaagaaaacaaaaacccccaggtcgctttattttgacctgtgttagggaccaaaaacggtggcagcactgtctagctgcgggcattagcctggaaaactagtgctctctgggtaaccactaaaatcccgaaagggtgggctttggggaccctccgaaccaatagatagcctccctcctcggacggggggcctgccc

SEQ ID NO: 32 - RNA, 305 nt, synthetic construct
  source 1..305: mol_type = other RNA
ttgctttcatagacccgtcttccgggagacgttaagaagatgcccgtggaaaatagtaggtagagttgtggcgtgacaacccacaactgcatctctttgcttatctagttacaatatatgttgacgtacaagaaggatcctgggaaacaggttcaacgggctcactgtggtggtgagccgtcgcatcacttgtatgtgctccaatattggttgtcgataagcgtcctgacatggctccatgcaacagcatgggggggtccagagtcagtcccctctttatttacctagagattcctctaggaatt

SEQ ID NO: 33 - RNA, 120 nt, synthetic construct
  source 1..120: mol_type = other RNA
accatggtcatgatgatgatagtgaaggacgctgaaagatgcgtagctaccctcctggtgcacttcctggtgcaaagcagaaccaaagggtacggtggtacggcggacagtagtcctgaa

SEQ ID NO: 34 - RNA, 117 nt, synthetic construct
  source 1..117: mol_type = other RNA
atggaggagccgcagtcagatcctagcgtcgagccccctctgagtcaggaaacattttcagacctatggaaactacttcctgaaaacaacgttctgtcccccttgccgtcccaagca

SEQ ID NO: 35 - RNA, 239 nt, synthetic construct
  source 1..239: mol_type = other RNA
gttgctcgactgtgaggggacctacccactgtgctgccacacaggaacttccaaccttcgggtggcgaggtagggcagaagagtgactgaacgaggatggtgtagagcaatggatggggggggagtccatggtgggctccggcgcgacgatgctaaaatctccatatcatgtgtggagtgggctgcttagtcgcttattagttgaaaattaggggggtccttagggacctctcccgccc

SEQ ID NO: 36 - RNA, 87 nt, synthetic construct
  source 1..87: mol_type = other RNA
gttgctcgactgtgaggggacctacccactgtgctgccacacaggaacttccaaccttcgggtggcgaggtagggcagaagagtgac

SEQ ID NO: 37 - RNA, 88 nt, synthetic construct
  source 1..88: mol_type = other RNA
ggtagaacacgtgggataggggatgaccttgtcgaccggttatcggtcccctgctccttcgagctggcaaggcgcccaaaggttctac

SEQ ID NO: 38 - RNA, 326 nt, synthetic construct
  source 1..326: mol_type = other RNA
actcgctcagagtcatcctaggctaggaccggccagacaaaggtccgacactacatgcagcgctctaggtgtgtagtgacagtaagcgcgctctatccgaaactccagtgacaggacaagaccccaggcgggacgccacacccatgtttgcagacatggcccgaggaaactctggtgtgggctggggggaatcctatgatcactggacggaaggtagagagttccagcacaacccctttagggtgggccgtaagtgcgtgggaacatttcctacagtctcactgagaagattggacggggtaccatgagtacccctcaccaggccc

SEQ ID NO: 39 - DNA, 20 bp, synthetic construct
  source 1..20: mol_type = other DNA
ccgtcgattgtccactggtc

SEQ ID NO: 40 - DNA, 20 bp, synthetic construct
  source 1..20: mol_type = other DNA
gaccagtggacaatcgacgg

SEQ ID NO: 41 - DNA, 35 bp, synthetic construct
  source 1..35: mol_type = other DNA
gcactggctgacagaccgtcgattgtccactggtc

SEQ ID NO: 42 - DNA, 35 bp, synthetic construct
  source 1..35: mol_type = other DNA
gaccagtggacaatcgacggtctgtcagccagtgc

SEQ ID NO: 43 - DNA, 70 bp, synthetic construct
  source 1..70: mol_type = other DNA
cgtactgctagctcgctgccatcgatgctgatgaggcactggctgacagaccgtcgattgtccactggtc

SEQ ID NO: 44 - DNA, 70 bp, synthetic construct
  source 1..70: mol_type = other DNA
gaccagtggacaatcgacggtctgtcagccagtgcctcatcagcatcgatggcagcgagctagcagtacg

SEQ ID NO: 45 - DNA, 105 bp, synthetic construct
  source 1..105: mol_type = other DNA
cgaatgcgatgctagtcgtagctagtccgatgatgcgtactgctagctcgctgccatcgatgctgatgaggcactggctgacagaccgtcgattgtccactggtc

SEQ ID NO: 46 - DNA, 105 bp, synthetic construct
  source 1..105: mol_type = other DNA
gaccagtggacaatcgacggtctgtcagccagtgcctcatcagcatcgatggcagcgagctagcagtacgcatcatcggactagctacgactagcatcgcattcg

SEQ ID NO: 47 - DNA, 140 bp, synthetic construct
  source 1..140: mol_type = other DNA
cgctgatgctgatcgtagctggatgctagtcgtagcgaatgcgatgctagtcgtagctagtccgatgatgcgtactgctagctcgctgccatcgatgctgatgaggcactggctgacagaccgtcgattgtccactggtc

SEQ ID NO: 48 - DNA, 140 bp, synthetic construct
  source 1..140: mol_type = other DNA
gaccagtggacaatcgacggtctgtcagccagtgcctcatcagcatcgatggcagcgagctagcagtacgcatcatcggactagctacgactagcatcgcattcgctacgactagcatccagctacgatcagcatcagcg

SEQ ID NO: 49 - DNA, 10 bp, synthetic construct
  source 1..10: mol_type = other DNA
tccactggtc

SEQ ID NO: 50 - DNA, 10 bp, synthetic construct
  source 1..10: mol_type = other DNA
gaccagtgga

SEQ ID NO: 51 - DNA, 20 bp, synthetic construct
  source 1..20: mol_type = other DNA
ccgtcgattgtccactggtc

SEQ ID NO: 52 - DNA, 20 bp, synthetic construct
  source 1..20: mol_type = other DNA
gaccagtggacaatcgacgg

SEQ ID NO: 53 - DNA, 35 bp, synthetic construct; identical to SEQ ID NO: 41
  source 1..35: mol_type = other DNA

SEQ ID NO: 54 - DNA, 35 bp, synthetic construct; identical to SEQ ID NO: 42
  source 1..35: mol_type = other DNA

SEQ ID NO: 55 - DNA, 70 bp, synthetic construct; identical to SEQ ID NO: 43
  source 1..70: mol_type = other DNA

SEQ ID NO: 56 - DNA, 70 bp, synthetic construct; identical to SEQ ID NO: 44
  source 1..70: mol_type = other DNA

SEQ ID NO: 57 - DNA, 100 bp, synthetic construct
  source 1..100: mol_type = other DNA
aatgataccgtaggagctcatgcggatatacgtactgctagctcgctgccatcgatgctgatgaggcactggctgacagaccgtcgattgtccactggtc

SEQ ID NO: 58 - DNA, 100 bp, synthetic construct
  source 1..100: mol_type = other DNA
gaccagtggacaatcgacggtctgtcagccagtgcctcatcagcatcgatggcagcgagctagcagtacgtatatccgcatgagctcctacggtatcatt

SEQ ID NO: 59 - DNA, 150 bp, synthetic construct
  source 1..150: mol_type = other DNA
agccaagcagtattcatcctgtacacaattccgataactatccctgatggaatgataccgtaggagctcatgcggatatacgtactgctagctcgctgccatcgatgctgatgaggcactggctgacagaccgtcgattgtccactggtc

SEQ ID NO: 60 - DNA, 150 bp, synthetic construct
  source 1..150: mol_type = other DNA
gaccagtggacaatcgacggtctgtcagccagtgcctcatcagcatcgatggcagcgagctagcagtacgtatatccgcatgagctcctacggtatcattccatcagggatagttatcggaattgtgtacaggatgaatactgcttggct

SEQ ID NO: 61 - DNA, 200 bp, synthetic construct
  source 1..200: mol_type = other DNA
aggacgactctggagtacatcttaggcggagaaccgtgatacacaatggaagccaagcagtattcatcctgtacacaattccgataactatccctgatggaatgataccgtaggagctcatgcggatatacgtactgctagctcgctgccatcgatgctgatgaggcactggctgacagaccgtcgattgtccactggtc

SEQ ID NO: 62 - DNA, 200 bp, synthetic construct
  source 1..200: mol_type = other DNA
gaccagtggacaatcgacggtctgtcagccagtgcctcatcagcatcgatggcagcgagctagcagtacgtatatccgcatgagctcctacggtatcattccatcagggatagttatcggaattgtgtacaggatgaatactgcttggcttccattgtgtatcacggttctccgcctaagatgtactccagagtcgtcct